European Patent Specification EP 3 567 111 B1, published July 9, 2025. Title: Gene for resistance to Beet Cyst Nematodea pathogen of the genus Heterodera. Applicant: KWS SAAT SE. The sequence listing filed with the application follows.

SEQUENCE LISTING (11 sequences)

SEQ ID NO: 1 - DNA, 4327 bp, Beta vulgaris
atggcagctgaagcaggtaatgtcaaatactgttggtcatttcttagagaagcggaagtggaggtatcccgcgtatatgatgacggttacctgtttttggaggaggatccagtggcatggattcaaagtcaccctgctgctgctgatcgtctctctgtgcgaatcttagagttgaaattggggctgaatggtgtggagaagataacagacatgatagaggagctgtctgagctcactcacctctatgtctatttgtgtcataacctcgattgtttgcctgacaccatcacaaggctgtccaaattaccagaaaatttggaagagctggagagccttacccatctctctcttccttattgtgtagatatcaagtcccttcctaatagtcttgcaaacctatccaacttgacgactttggatcttattggatgccattcccttacagaattgcctccaaatttgaatgttgtacacctcattattaaacgttgctgcaaaatcaaggcccttcctacaggtttaaataacctggccagcttacatctcaaacaatgtaactattgtcttgccaatttaaagcactcgctcaacctacgccacctcacccttcagagttgcgattttcattctcacgctgacgttatagaattcctgccaaatttggatgagctgctacaattatctcttcttgatatccaggataccaaaatcagatatcttccttggagcatcacaaagctactcaatttgaaatttctatgtctccctcggggttttatactcgaaacactaccatatcatctgaatgattccgtcatcatttatatgaaggattgtcacgatcgcaaaacttggaaagaactcaaaacagagattcaaggtaagtgtttccgctatttatctcacgaattattgtttcatgttcgcttctcttccggcagggccgtcttgaagattttgggggccggattctaacatgaaaattgggcccctaaatttatagaaaataaagatggaagattaaagttctaaagatggaaagttgaaaatgaagataaatcattgacaaatttattataggtgggaaacaagggtgatttcttcaaatataaagtaaaattttcaaaacaatatattttggggcctttataattttggaggccatgtgcaattgggctctttgcacaccctcatctacccctctgtcttccggtaaatagcaaatagcaaatagcatcgccctctttttatcgcaatatgcaaacatgggaaagttatatttcaaatgtatatattcataattcaagcattgttgtttcatgttctcctttctataccaaaatgtttgtttgtcctcctaatccaagtccaaccaattatgcaaataaggaaagattagattcagactatatataataatgttaatatattttcctgttcttcaattttatttcttaattatcttcctctttgtcctcctccagtggataatttgggaatatcaatgtctgtacctcggaactcctcttgttacctttggttggactccaacaagagcctacatccatggctgcagaataattacgattttcaaccgtctgtgaaattcctcgatttaaattttttggatgatgagtttggagatctcacgttgctgaaagagctcacacatgtgacacatctctatatttctggtcatgtagacctctgccgcctccctgacacactcacaaatattacccatctctctcttcatactgaagatgacactgatgattcatttgattcctttcttgataggctggcagagccatcaaacttggtatctttagatgtagatcttagtgaaacatacttgccgtcaaacatccatcaattcgtcaaccttaaatgtctcactgtaagatatgccaacagcaagccattagtacctgataactgggaaaagctatctaatttgaaatctttggttctctatacatgttataatgtatcattgccaacacatttgaatctcactaacctcaagcttttcaattgctttttcgagaatgtcagcttactacctacaagtctacaccgcctagaattattgcatagcaacgactattgcagtgccttttgctgtgatgacggggattgtagtgaagagcctatactatgcttgaatcagtttgtcaacctagagacgctctctataacatgttacgagtacactggcacccgacttcccagcatagcaggactacgcaacttgaaagaattacaacttaaggattgtttcggcctcaaagaattacccccagatttggatgagctagtggaattatccattctcaatatcagcggtaccagagtcaagtcctttcctgattgcatcacaaagctacaaaagttgaaacacgtagtcctgcccaagtgcttcaaaaaggaaaatttacccaataattcaaaaacgaagtacaccactgatgacacggatgaagaatactacaagcatagaggctattatagtagtgaatatgaaacctcaaatataacctctgatgaaagtaatgagatcacagtagtagattctgcagaggtagccgacaaagtggtttcagaatattcacaggaaggcatcatttcgcagcagatatcatcaccccaactcctgagtatacctaatgctaatcagtttcttggaggtacgtgcttctactatttcagaaatcattgtgtggagtacattgcaattcttctatcttaaaatcagaatctaattgtcaaatgatcaaggtagtgtgcttccaagttccaacactccttaaccccattaatggggtctgatagagtttgtttcattatattaacttttattgcgtgggtttgaatattaagtttttttatacaagcagatactcatttcaatggtagaagcaatacgatgggcgagaattcacaagttcaagagatggaaacttcatctacaggactcaattcaaatacaaatgaaataaatgtcaccgaccagatgttggaattcctatttgggaactcatcatttgattttgggcacatttcttatagtgatgtgactaatattgatcgtgttgagaataacgatcatgcttcagaatatacgcagaacaacgagaatccaccaagtgatgagaaccagggaaagagacagaagaaggagattactcatgagaaaaatccatgtctgatggataaaaacatgacacatgaggagctaggcggtatgttttatcctttacaaagtattttctcagttctcttttaaattcagaagtatatcgtgatatgcttactgtgactggtgattatcaactatttaaaaagcaaagtttgattttgacaagaataaatgggaactccattaatttaaaagattctgcttttggtgcgaatagaatttaatcacaatggaggagaggatgcagtttatgagatcagtcacagcgcttcttgcggttcaccggaccaagacatggagaatatgcctgtaggaaatgataaagattcaacatccaccatagttcgccgagggaaacgtaacaaaatagagtttaatttgactagagaggaacttgaatcatactggtccagaaacatgacggtagaagatgttgcaaaagacataggtggtatgtttccattctctacaaactatacggtcattcactgcatttaattgatagatgcatttgatgttatatgattcattccagtgtcaaggtctacatttaaacgctggttgaaggcctccggtattaaatggcaaacaagcaggatttcgaaaagtcaatgtgccaacaacaagaataccaatactgcatcattctctggaagtaaacctgcagaggtcaactgtcatgaacatgcacctgagtgtttaagtgatgcaaatgaatgtgatgtcgttaacaacttaacccttgctgtgacaatggatactgaggaagagcctggagtagcaacgcaatgccatagcaatggtagcaaacaggcctctgacactctggtgggtgcagatcagggtactcaacaagagagtccaagtttaagcaaaatcattgtgaaagccacttacaaagatgatactgttagatttcatatctcttcaactgctagtttccatgaactagaaaaagaagtggcaaaaaatctaaaactcaagctaagcaaatttaaaataaaatatcaagatgaggacaaagagttgatgctaatgaccttggactctcacttgaaggaacttctcgatctttcaaaatcatctggtagcaaaattgttcggttgttaatatttgatttgtga

SEQ ID NO: 2 - DNA, 3255 bp, Artificial Sequence
  cDNA of LRR2
atggcagctgaagcaggtaatgtcaaatactgttggtcatttcttagagaagcggaagtggaggtatcccgcgtatatgatgacggttacctgtttttggaggaggatccagtggcatggattcaaagtcaccctgctgctgctgatcgtctctctgtgcgaatcttagagttgaaattggggctgaatggtgtggagaagataacagacatgatagaggagctgtctgagctcactcacctctatgtctatttgtgtcataacctcgattgtttgcctgacaccatcacaaggctgtccaaattaccagaaaatttggaagagctggagagccttacccatctctctcttccttattgtgtagatatcaagtcccttcctaatagtcttgcaaacctatccaacttgacgactttggatcttattggatgccattcccttacagaattgcctccaaatttgaatgttgtacacctcattattaaacgttgctgcaaaatcaaggcccttcctacaggtttaaataacctggccagcttacatctcaaacaatgtaactattgtcttgccaatttaaagcactcgctcaacctacgccacctcacccttcagagttgcgattttcattctcacgctgacgttatagaattcctgccaaatttggatgagctgctacaattatctcttcttgatatccaggataccaaaatcagatatcttccttggagcatcacaaagctactcaatttgaaatttctatgtctccctcggggttttatactcgaaacactaccatatcatctgaatgattccgtcatcatttatatgaaggattgtcacgatcgcaaaacttggaaagaactcaaaacagagattcaagtggataatttgggaatatcaatgtctgtacctcggaactcctcttgttacctttggttggactccaacaagagcctacatccatggctgcagaataattacgattttcaaccgtctgtgaaattcctcgatttaaattttttggatgatgagtttggagatctcacgttgctgaaagagctcacacatgtgacacatctctatatttctggtcatgtagacctctgccgcctccctgacacactcacaaatattacccatctctctcttcatactgaagatgacactgatgattcatttgattcctttcttgataggctggcagagccatcaaacttggtatctttagatgtagatcttagtgaaacatacttgccgtcaaacatccatcaattcgtcaaccttaaatgtctcactgtaagatatgccaacagcaagccattagtacctgataactgggaaaagctatctaatttgaaatctttggttctctatacatgttataatgtatcattgccaacacatttgaatctcactaacctcaagcttttcaattgctttttcgagaatgtcagcttactacctacaagtctacaccgcctagaattattgcatagcaacgactattgcagtgccttttgctgtgatgacggggattgtagtgaagagcctatactatgcttgaatcagtttgtcaacctagagacgctctctataacatgttacgagtacactggcacccgacttcccagcatagcaggactacgcaacttgaaagaattacaacttaaggattgtttcggcctcaaagaattacccccagatttggatgagctagtggaattatccattctcaatatcagcggtaccagagtcaagtcctttcctgattgcatcacaaagctacaaaagttgaaacacgtagtcctgcccaagtgcttcaaaaaggaaaatttacccaataattcaaaaacgaagtacaccactgatgacacggatgaagaatactacaagcatagaggctattatagtagtgaatatgaaacctcaaatataacctctgatgaaagtaatgagatcacagtagtagattctgcagaggtagccgacaaagtggtttcagaatattcacaggaaggcatcatttcgcagcagatatcatcaccccaactcctgagtatacctaatgctaatcagtttcttggagatactcatttcaatggtagaagcaatacgatgggcgagaattcacaagttcaagagatggaaacttcatctacaggactcaattcaaatacaaatgaaataaatgtcaccgaccagatgttggaattcctatttgggaactcatcatttgattttgggcacatttcttatagtgatgtgactaatattgatcgtgttgagaataacgatcatgcttcagaatatacgcagaacaacgagaatccaccaagtgatgagaaccagggaaagagacagaagaaggagattactcatgagaaaaatccatgtctgatggataaaaacatgacacatgaggagctaggcgaatttaatcacaatggaggagaggatgcagtttatgagatcagtcacagcgcttcttgcggttcaccggaccaagacatggagaatatgcctgtaggaaatgataaagattcaacatccaccatagttcgccgagggaaacgtaacaaaatagagtttaatttgactagagaggaacttgaatcatactggtccagaaacatgacggtagaagatgttgcaaaagacataggtgtgtcaaggtctacatttaaacgctggttgaaggcctccggtattaaatggcaaacaagcaggatttcgaaaagtcaatgtgccaacaacaagaataccaatactgcatcattctctggaagtaaacctgcagaggtcaactgtcatgaacatgcacctgagtgtttaagtgatgcaaatgaatgtgatgtcgttaacaacttaacccttgctgtgacaatggatactgaggaagagcctggagtagcaacgcaatgccatagcaatggtagcaaacaggcctctgacactctggtgggtgcagatcagggtactcaacaagagagtccaagtttaagcaaaatcattgtgaaagccacttacaaagatgatactgttagatttcatatctcttcaactgctagtttccatgaactagaaaaagaagtggcaaaaaatctaaaactcaagctaagcaaatttaaaataaaatatcaagatgaggacaaagagttgatgctaatgaccttggactctcacttgaaggaacttctcgatctttcaaaatcatctggtagcaaaattgttcggttgttaatatttgatttgtga

SEQ ID NO: 3 - protein, 1084 aa, Beta vulgaris
MAAEAGNVKYCWSFLREAEVEVSRVYDDGYLFLEEDPVAWIQSHPAAADRLSVRILELKLGLNGVEKITDMIEELSELTHLYVYLCHNLDCLPDTITRLSKLPENLEELESLTHLSLPYCVDIKSLPNSLANLSNLTTLDLIGCHSLTELPPNLNVVHLIIKRCCKIKALPTGLNNLASLHLKQCNYCLANLKHSLNLRHLTLQSCDFHSHADVIEFLPNLDELLQLSLLDIQDTKIRYLPWSITKLLNLKFLCLPRGFILETLPYHLNDSVIIYMKDCHDRKTWKELKTEIQVDNLGISMSVPRNSSCYLWLDSNKSLHPWLQNNYDFQPSVKFLDLNFLDDEFGDLTLLKELTHVTHLYISGHVDLCRLPDTLTNITHLSLHTEDDTDDSFDSFLDRLAEPSNLVSLDVDLSETYLPSNIHQFVNLKCLTVRYANSKPLVPDNWEKLSNLKSLVLYTCYNVSLPTHLNLTNLKLFNCFFENVSLLPTSLHRLELLHSNDYCSAFCCDDGDCSEEPILCLNQFVNLETLSITCYEYTGTRLPSIAGLRNLKELQLKDCFGLKELPPDLDELVELSILNISGTRVKSFPDCITKLQKLKHVVLPKCFKKENLPNNSKTKYTTDDTDEEYYKHRGYYSSEYETSNITSDESNEITVVDSAEVADKVVSEYSQEGIISQQISSPQLLSIPNANQFLGDTHFNGRSNTMGENSQVQEMETSSTGLNSNTNEINVTDQMLEFLFGNSSFDFGHISYSDVTNIDRVENNDHASEYTQNNENPPSDENQGKRQKKEITHEKNPCLMDKNMTHEELGEFNHNGGEDAVYEISHSASCGSPDQDMENMPVGNDKDSTSTIVRRGKRNKIEFNLTREELESYWSRNMTVEDVAKDIGVSRSTFKRWLKASGIKWQTSRISKSQCANNKNTNTASFSGSKPAEVNCHEHAPECLSDANECDVVNNLTLAVTMDTEEEPGVATQCHSNGSKQASDTLVGADQGTQQESPSLSKIIVKATYKDDTVRFHISSTASFHELEKEVAKNLKLKLSKFKIKYQDEDKELMLMTLDSHLKELLDLSKSSGSKIVRLLIFDL

SEQ ID NO: 4 - DNA, 8671 bp, Beta vulgaris
atggtttctgcgggtgtaattcgttttgtagctgggattattggtaagtatattcacaaactatcttgctctattaaattacaaataagaaaaatgaagtatttattcttcaacgaatgtaatatgttctaacttatatgtattaatttctttccttgcaatattgtaattaataaagttggtttattttggtttgcaggtaatatgacagcttttttcttattcttgtctccagtgtaagttattcatgatggatttgcttcgtactatattcatgtgcataatttacaatatatgaagatgaagctatataatgtgtacccctctcttgcttatgcaatggaaggaatcattattattcattatagtaggtatttatgaaaattctataatttggagtacagatttgtaataaaaagatttaaactaatgaattcaatcaaaagcttaagctgatggttagagtcccacgaatagttttatactctatcacacccccctcacgcgagatcccattgagcttaaagtgtggatgtagcgtaggtctccctcatactagacatattccacttagaaagaaggggtggacgagatttgaacccgtgacatttatgtcacgttggctctgataccatgtcaaaggaccaactcaaccaagagcttaagcttatggttggagactggagtcccaaaaatagttttatactatgtcggttatatttgcacatgattttcattcttgctttccatcttttaggccaacattcatcggaatatgcaagaagaagacggtggaacaatactcgccagtgccatacttagccacatttgtgaattgcatgctttgggttgtgtatggtctgcctattattcaccctaatagcattttagtggtgacaatcaatggagctgggttttttattgaactgctttacttgatactcttcgtgctttactctgacaaaaagaataggctcaaaattgtgttgattgcaattattgagatcgtaattgtgggaattatgactaccttggtcctcaactttgttcatactaccaagcgtaggtcttcaattgttggtatgattgccatcatatgtaacatcatgatgtatgcctctcctttatccgtcttggtaattatgcttaattaatctccctttctctttactacttgctaacaagtacgcggaactagaattattttctaaattacttaatatttcctccgtttcaaattaaatgcaacagcttctaaaaacgacagtttcaaattaaatgcaacgttttacttctttctattcttggtaaagactttttagtgtgaaattacagatataaccttactaaaacaaattaagcgttattaacttagtcacatgtccttactttttcttaatctcacctaagaagttttgcctaagagaatgtatcatctaaatcgttacatttaatttggaacagaggaaataatataaatccctaattttgtgtttttggacagaaattggtgataacaacaaaaagcgtggaatacatgccgttatctttatcaattgcttcatttgctaatggcattgcatggacagtctatgctttgtatcctttcgatccttacattgccgtaagcctccctttgacccttaaattgcaaataaattacatattgcaagttctaagatttttattgtttgtaataaatttgacatgctaattattagattcctcgttctattagcttatattgtgtatgtgtagtattgcatctaccaaaatatccttctaaattcacaaatcaatgcataatcaaaaatattaaatcatataaaagaaaatcaaccatgcaggtagatattgttgtatagcgatatattttacttaatttaagacgtttgatgaattttttttcgctacagtatgttactctcattatatacttcgttcgtttcgttttaaatgcaacaaagcggtattttttatgagatataaaatatttattcgttgcatttaaaacgaaacggaagaagtaatcagaaaagactagtaaatagtacgagctaaagaaaatggcttttgttttacaacacaggcaccaaatgggctgggtacactatttgcagtggtccaactgattctgtatgcaacatactacaagtccacaaaagagcagatggcagcaagaaaagccaaaaatgcagtgggcctgactgaagttgtcttcaacggagactctggaaaaatgggccaagtaccacataatagtcgggcccaaatcccttgaagcccaatccaattttagctcatgggttcccaagctcacccggctgatcaaattcctttttttcctttttcttgcttctcatgaattctccttactattatcaaccaataaaacatggagtcatttatggaatttttttttttctttttgttgaatagaattattaactgaaataatgttgttttgtcatctataatctcgattagttttagcttaatgacaagatattgaatggtctttggattgaacggttgattaatgatatacttcttccgttttgaattactccgttatttatttatgagatttgaccatatattatttacaattagataaaatcaaatgttataatgtaatatgttgttggattgtctcaatgtatattttcataaaatcaaatttttggtgtccccccctcttcccttatataatagagatgattcgaattcaacaatattgctatataattaaattgtttgcctcgaagttacgaacttaaaattgaacaaatcaatctatttcaactttcaagcatagaaagttgaaatacagaacaaaacaagtcccccaattggaaaatatgaatttgaatctagcttcaaaatctacacatagtcgtttctaatgttgaaattgaggggaagataaatcgtactgtactaattgtctaattgaaacaataaacaaaatcaattggttattcaacatatctataaactcagctgaataaacattaacatattcaaacactgcacaaaatcataataagtattcaaattgaacacaatcaaaattcatcaaaaaaattcatataacgactctgtttggggaagtattttagctaccttaaatgattaggtgctaacatattttaggtactaaaataattagtagtgtttggggagcccctaaaataaatttcaggcgactaaaatgacttaaatgataagttaaaaattttaccttttcaaaatcaggtgattgaaattttggaaaatctttccaaaattttgacaacaattaattttgctaaaataatttattgacttaatcaactaatattgctaaacagttaaactaatcaattaccttatggattcaaggcttctaacaccttatcttttattttcagctaataatgctaaacagagccaaacaactgatttatcaattacaatacagagattcaaacctcctttcatttccctaatcaactgaaaataagccctagaaaacgaaacctaaccaccgaaaccgtaaagatatcaagtttctgtgcctctttgctccaccctttcccaaaccctaacctccctttcctctttctgacattttctctctcctctttctgggttttcttctttctgtgattttttcagtttgaattgttttgggttgtggatgtgaatgttgtgggaatggagaaagaagaggtgggtgattatatagtgaatggattgttgaaatcttgagatttggttttgatactagagtaaagcaagctcctccatagtccatagtccatagccctgaaaaaaaaaaaaaaagaggtcctccattgaagagagtaaagtagcatctgcaaaataatagtagagttttagatctaatttcttcaattttacgccttttgataatggcagctgaagcagtaggtaatgtcaaatactgtcggtcatatcttagaggagtagatgtcgaagtatcccgcgtatatgatgacggttacctgtttttggaggaggatccagtggcatggattgaaagtcacccagctgctgctgatcgtctctctgtgcgaatcttggagttgaaatggatggatgatgtggataagataacagacatgataggggagctgtctgagctcactcacctctatttctattggtgtccaaacctcaagtctttgactgacaccatcacaaggctgtccaacttacagttgttaaaacttgaaggttgttataaactggaagaattaccagaaaatttgggagagctggagagccttacccatctctctatttcttcttgtagagatatcaagtcccttcctaatagtcttacaaacctatccaacttgacgactttggatctttttggatgcgattcccttacagaattgcctccaaatttaaacgttatacacctcattattaaacattgctgcagcatcaaggcccttcctacaggtttaagtaacctggccagcttacatctcaaacaaagtcactattgtcttgccaatttaaaggactcgctcaacctacgccaccttacccttgagagttgtgattttcatggtcacgctaacgttatagaattcctgccaaatttggatgagctgctacaattatctcttgtggatatccaggataccaaagtcagatatcttccttggagcatcacaaagttactcaatttgaaaattctatgtctccccggggactttatacttgaaacactaccatatcatttgaatgattccgtcatcatttctatgaaggattgtcacaatcgcaaaacttggaaagaactcaaaacagagattcaaggtaagtgttttcgctattatctcacgaattgttgtttcatgtaatgtttgcttctcttccggtaaatagcaaatagcaaatagcatagccctctttttatgtcaagaaacttattcgtaccattgtgcaaacatgggatggaactgggaaggttatatttcaagcattgttgtttcatgctctccttttctatccctaacggcccctttggttagtggttataaatagtggtaatggtaatgaaatttagtgtaaatttgtaaagattttcacatgtccataaccatgggaatgaaactttatcacaaaacatgggttttcctttataaatttttattaccaccttcccaagtggtaatggatagtaatgagattttaggaagaaaatggatatcttgtgattaagtagcattaccattggtaatgacattggatttctagcacaaatttacactataatgcattaccattcacatcatttataacctcttaccaaacgggccgttaaaagtttatttgtcctcctagtccaaccaattatgcaaaataaggagagattaaattcagactatacatactgttcatatattttcctgttcttcaattttatttcttaattatcttcctctttgtgctcctcctccagtgaaaaatttgggaatatcaatgtctgtacctcggaacccctcttgttacctttggttggacaccaacaagaaactacatccatggctgcagaataattaccatcgtcaaccgtttgtgaaatccctgcatttgcaatttttggatgatgagtttggagatctcaagttgttgaaagagctcacacatgtgacacatctctatatttctggtgatgtagaccactgccgcctccctgacacactcacaaatattacccatctctctcttcatcattgttacacttacactgatgattcatttaagtccttattactcgatagcctggcagagccatcaaacttggtatctttagatgtagatcttagtgaaacatacttgccgtcgaacatccatcaattcgtcaaccttaaatgtctcactgtaagaaatgaccacagcgagcaattagtacctgatgactgggaaaagctatctaatttgaaatctttggttctctacagatgttatgatgtatcattgccaacacatttgaatctcaccaacctcaagctttttgattgctttttcaagaatgtcagcttactacctacaagtatacaccgcctagaattatggcatagcaaatacttttgctgtaaaaacaggtattgtagtaaagagcctatagtatgcttgaatcagttggtcaacctaaagacgctctcaataacatgttacaagtacactagcaacctacttcccagcatagcaggactacgcaacttgaaagaattacaacttaaggattgtttcggcctcaaagaattacccccagatttggatgagctagtggaattatccattctcaatatcagcggtaccagagtcaagtcctttcctgattgcatcacaaagctacaaaagttgaaacacgtagtcctgcccaagtgcttcaaaaaggaaaatttaccaattaatttcgaaacgacgtatgatgtcacggatgaagagtactacgagaatagaggctattatgatagtgactatgatacattctctgatgatgaaagcaatgagttcgcagtagtagattctgcagagtcagccgacgaactggtttcagaatattcacaggaaggcattattgctcagcagatatcagctaatgctaatgtcaatcagcttcttggaggtacgtgcttctactatttcagaaatcatagtgtggagtacattgcaattcttctattttaaaatcagaatctaattgtcaaatgatcaaggtagtgtgcttccaagttccaacactccttaaccccattaatggggtctgaaccgtctgatagagtttgtttcataatattaacttttattgcgtgggtttgaatattaagtttttttatacaagcagatactcatttcaatggtagaagcaataccatgggcgagagttcacaagttcaagagatggaaacttcatctacaggactcaattcatatacaaatgaaataaatctcaccgaccagatgtcggaattcgaattaattgagatctcatcatttgattttgggcctatttcctcttgtgatgtaaataatattgctggtgttgagaacaaccataatgcttcagaatatacacagaacaacgagaattcaccaagtgatgagaaccagggaaagagacaggaggagattattcatgagaaaaatccatgtctgaatctgatggataaaattatgacacaggtgaaccttggcaaggagctaggtggtacgtttttatcctttacaaagtattttctcagtcctcttttgaattcagaatatgattaccatgagtatgattttcttgtattgatgaatattaatttttttcatacaagcagatactcatttcaatggtagaagcaatacaattggcgagagttcacatgatgaagagatggaaacttcatctacaggactcaattcagatacacatgaaataaatccacaaagtggtgataagcagcgaaagagacagaagaaggagattacccgtgagaaaaatgcatgtcttcttggcaaggagctaggtggtacgtttttatcctttacatagtatttcctccgtcctcttttaaattcagaagcatatcgtgatatgcttccgtgactatgggtttcttgtatattatattggtgattattaactatttaaacagcaaagtttgattttgacaagaataagtaggaactttaaaagattttgtttttggtgcaaatagaatttaatcacaatggacgagaagatgcagttgatgggatcagtcaccgcgcttctttgggtctaccagaccaagacatggagaatatgcctgtaggaaatgataaagattcaacatccaccatagttcgccgagggaaacgtaacaaaatagagtttaatttgactagagagcaacttcaatcatactggtccagaaacatgacggtagaagatgttgcactagaattacgtggtatgtttccattctctgcaaactatacggtcattcactgcacttaattgatagatgcatttgatgttatatgattcattccagtggcaaggtcttcatttagacgctggttgacggcctccgaaattccatggcaaacaagcaggatttcgaaaagtcaatgtgccaacaacaagaataccaatactgcatcatcctctggaagtaaacctgcagaggtcaatttagtgaaaccctttaatactccaactggtcatgaacatgcacctgagtgtttaagtgatgcaaacgaatgcgttgtcgttaacaacttcagccttgctgtgacgacggacgctgagggagagcctggagtagcaacgagatgccatagcaatggtcgtgaacaagcttctgacgctttggtgggtacaaatcagggtactcgacaagagagcccaagtttaagcaaattcgttgtgaaagccacttataaagatgatgattatagaattgagttaccttcaactgctagtttccatgaactaaagaaagaagtggctcggactctagaacttgagatgtgcaaattcaaaataagatataaggacgaggataacgagtggacgcgaatgagcattgactctcatttaaagcatcttatggatctttcaagatcatctggtaaaaatgttattcggttgtcagtaattgatttgtga

SEQ ID NO: 5 - DNA, 4290 bp, Artificial Sequence
  cDNA of LRR1
atggtttctgcgggtgtaattcgttttgtagctgggattattggtaatatgacagcttttttcttattcttgtctccagtgccaacattcatcggaatatgcaagaagaagacggtggaacaatactcgccagtgccatacttagccacatttgtgaattgcatgctttgggttgtgtatggtctgcctattattcaccctaatagcattttagtggtgacaatcaatggagctgggttttttattgaactgctttacttgatactcttcgtgctttactctgacaaaaagaataggctcaaaattgtgttgattgcaattattgagatcgtaattgtgggaattatgactaccttggtcctcaactttgttcatactaccaagcgtaggtcttcaattgttggtatgattgccatcatatgtaacatcatgatgtatgcctctcctttatccgtcttgaaattggtgataacaacaaaaagcgtggaatacatgccgttatctttatcaattgcttcatttgctaatggcattgcatggacagtctatgctttgtatcctttcgatccttacattgccgcaccaaatgggctgggtacactatttgcagtggtccaactgattctgtatgcaacatactacaagtccacaaaagagcagatggcagcaagaaaagccaaaaatgcagtgggcctgactgaagttgtcttcaacggagactctggaaaaatgggccaatttgaattgttttgggttgtggatgtgaatgttgtgggaatggagaaagaagaggtggctgaagcagtaggtaatgtcaaatactgtcggtcatatcttagaggagtagatgtcgaagtatcccgcgtatatgatgacggttacctgtttttggaggaggatccagtggcatggattgaaagtcacccagctgctgctgatcgtctctctgtgcgaatcttggagttgaaatggatggatgatgtggataagataacagacatgataggggagctgtctgagctcactcacctctatttctattggtgtccaaacctcaagtctttgactgacaccatcacaaggctgtccaacttacagttgttaaaacttgaaggttgttataaactggaagaattaccagaaaatttgggagagctggagagccttacccatctctctatttcttcttgtagagatatcaagtcccttcctaatagtcttacaaacctatccaacttgacgactttggatctttttggatgcgattcccttacagaattgcctccaaatttaaacgttatacacctcattattaaacattgctgcagcatcaaggcccttcctacaggtttaagtaacctggccagcttacatctcaaacaaagtcactattgtcttgccaatttaaaggactcgctcaacctacgccaccttacccttgagagttgtgattttcatggtcacgctaacgttatagaattcctgccaaatttggatgagctgctacaattatctcttgtggatatccaggataccaaagtcagatatcttccttggagcatcacaaagttactcaatttgaaaattctatgtctccccggggactttatacttgaaacactaccatatcatttgaatgattccgtcatcatttctatgaaggattgtcacaatcgcaaaacttggaaagaactcaaaacagagattcaagtgaaaaatttgggaatatcaatgtctgtacctcggaacccctcttgttacctttggttggacaccaacaagaaactacatccatggctgcagaataattaccatcgtcaaccgtttgtgaaatccctgcatttgcaatttttggatgatgagtttggagatctcaagttgttgaaagagctcacacatgtgacacatctctatatttctggtgatgtagaccactgccgcctccctgacacactcacaaatattacccatctctctcttcatcattgttacacttacactgatgattcatttaagtccttattactcgatagcctggcagagccatcaaacttggtatctttagatgtagatcttagtgaaacatacttgccgtcgaacatccatcaattcgtcaaccttaaatgtctcactgtaagaaatgaccacagcgagcaattagtacctgatgactgggaaaagctatctaatttgaaatctttggttctctacagatgttatgatgtatcattgccaacacatttgaatctcaccaacctcaagctttttgattgctttttcaagaatgtcagcttactacctacaagtatacaccgcctagaattatggcatagcaaatacttttgctgtaaaaacaggtattgtagtaaagagcctatagtatgcttgaatcagttggtcaacctaaagacgctctcaataacatgttacaagtacactagcaacctacttcccagcatagcaggactacgcaacttgaaagaattacaacttaaggattgtttcggcctcaaagaattacccccagatttggatgagctagtggaattatccattctcaatatcagcggtaccagagtcaagtcctttcctgattgcatcacaaagctacaaaagttgaaacacgtagtcctgcccaagtgcttcaaaaaggaaaatttaccaattaatttcgaaacgacgtatgatgtcacggatgaagagtactacgagaatagaggctattatgatagtgactatgatacattctctgatgatgaaagcaatgagttcgcagtagtagattctgcagagtcagccgacgaactggtttcagaatattcacaggaaggcattattgctcagcagatatcagctaatgctaatgtcaatcagcttcttggagatactcatttcaatggtagaagcaataccatgggcgagagttcacaagttcaagagatggaaacttcatctacaggactcaattcatatacaaatgaaataaatctcaccgaccagatgtcggaattcgaattaattgagatctcatcatttgattttgggcctatttcctcttgtgatgtaaataatattgctggtgttgagaacaaccataatgcttcagaatatacacagaacaacgagaattcaccaagtgatgagaaccagggaaagagacaggaggagattattcatgagaaaaatccatgtctgaatctgatggataaaattatgacacaggtgaaccttggcaaggagctaggtgatactcatttcaatggtagaagcaatacaattggcgagagttcacatgatgaagagatggaaacttcatctacaggactcaattcagatacacatgaaataaatccacaaagtggtgataagcagcgaaagagacagaagaaggagattacccgtgagaaaaatgcatgtcttcttggcaaggagctaggtgaatttaatcacaatggacgagaagatgcagttgatgggatcagtcaccgcgcttctttgggtctaccagaccaagacatggagaatatgcctgtaggaaatgataaagattcaacatccaccatagttcgccgagggaaacgtaacaaaatagagtttaatttgactagagagcaacttcaatcatactggtccagaaacatgacggtagaagatgttgcactagaattacgtgtggcaaggtcttcatttagacgctggttgacggcctccgaaattccatggcaaacaagcaggatttcgaaaagtcaatgtgccaacaacaagaataccaatactgcatcatcctctggaagtaaacctgcagaggtcaatttagtgaaaccctttaatactccaactggtcatgaacatgcacctgagtgtttaagtgatgcaaacgaatgcgttgtcgttaacaacttcagccttgctgtgacgacggacgctgagggagagcctggagtagcaacgagatgccatagcaatggtcgtgaacaagcttctgacgctttggtgggtacaaatcagggtactcgacaagagagcccaagtttaagcaaattcgttgtgaaagccacttataaagatgatgattatagaattgagttaccttcaactgctagtttccatgaactaaagaaagaagtggctcggactctagaacttgagatgtgcaaattcaaaataagatataaggacgaggataacgagtggacgcgaatgagcattgactctcatttaaagcatcttatggatctttcaagatcatctggtaaaaatgttattcggttgtcagtaattgatttgtga

SEQ ID NO: 6 - protein, 1429 aa, Beta vulgaris
MVSAGVIRFVAGIIGNMTAFFLFLSPVPTFIGICKKKTVEQYSPVPYLATFVNCMLWVVYGLPIIHPNSILVVTINGAGFFIELLYLILFVLYSDKKNRLKIVLIAIIEIVIVGIMTTLVLNFVHTTKRRSSIVGMIAIICNIMMYASPLSVLKLVITTKSVEYMPLSLSIASFANGIAWTVYALYPFDPYIAAPNGLGTLFAVVQLILYATYYKSTKEQMAARKAKNAVGLTEVVFNGDSGKMGQFELFWVVDVNVVGMEKEEVAEAVGNVKYCRSYLRGVDVEVSRVYDDGYLFLEEDPVAWIESHPAAADRLSVRILELKWMDDVDKITDMIGELSELTHLYFYWCPNLKSLTDTITRLSNLQLLKLEGCYKLEELPENLGELESLTHLSISSCRDIKSLPNSLTNLSNLTTLDLFGCDSLTELPPNLNVIHLIIKHCCSIKALPTGLSNLASLHLKQSHYCLANLKDSLNLRHLTLESCDFHGHANVIEFLPNLDELLQLSLVDIQDTKVRYLPWSITKLLNLKILCLPGDFILETLPYHLNDSVIISMKDCHNRKTWKELKTEIQVKNLGISMSVPRNPSCYLWLDTNKKLHPWLQNNYHRQPFVKSLHLQFLDDEFGDLKLLKELTHVTHLYISGDVDHCRLPDTLTNITHLSLHHCYTYTDDSFKSLLLDSLAEPSNLVSLDVDLSETYLPSNIHQFVNLKCLTVRNDHSEQLVPDDWEKLSNLKSLVLYRCYDVSLPTHLNLTNLKLFDCFFKNVSLLPTSIHRLELWHSKYFCCKNRYCSKEPIVCLNQLVNLKTLSITCYKYTSNLLPSIAGLRNLKELQLKDCFGLKELPPDLDELVELSILNISGTRVKSFPDCITKLQKLKHVVLPKCFKKENLPINFETTYDVTDEEYYENRGYYDSDYDTFSDDESNEFAVVDSAESADELVSEYSQEGIIAQQISANANVNQLLGDTHFNGRSNTMGESSQVQEMETSSTGLNSYTNEINLTDQMSEFELIEISSFDFGPISSCDVNNIAGVENNHNASEYTQNNENSPSDENQGKRQEEIIHEKNPCLNLMDKIMTQVNLGKELGDTHFNGRSNTIGESSHDEEMETSSTGLNSDTHEINPQSGDKQRKRQKKEITREKNACLLGKELGEFNHNGREDAVDGISHRASLGLPDQDMENMPVGNDKDSTSTIVRRGKRNKIEFNLTREQLQSYWSRNMTVEDVALELRVARSSFRRWLTASEIPWQTSRISKSQCANNKNTNTASSSGSKPAEVNLVKPFNTPTGHEHAPECLSDANECVVVNNFSLAVTTDAEGEPGVATRCHSNGREQASDALVGTNQGTRQESPSLSKFVVKATYKDDDYRIELPSTASFHELKKEVARTLELEMCKFKIRYKDEDNEWTRMSIDSHLKHLMDLSRSSGKNVIRLSVIDL

SEQ ID NO: 7 - DNA, 3773 bp, Beta vulgaris
atggcagatgaagcaggtaatgtcaactactgttggacgtgttggtcatctattagaaaagtggaagtcgaagtatcccgcatatatgatgacggttacctgttattgaaggaggatccagtggcatggattcaaagtcaccccgctgctgctgatcgtctctctgtgcgaatcttggagttgacattggagctgtatggtgtggataagataacagacatgataggggagctgtctgagctcactcacctctatttctattggtgtctttacctaaagtgtttgcctgacaccatcacaaggctgtccaacttacagttgttaaaacttgtaggttgttatgaattggaagaattaccagaaaatttgggagagctggagagccttacccatctctctctttctcagagtcaaggtatcaagtcccttcctaatagtcttacaaacctatccaacttgacaactttgaatatttttcaatgcaattcccttacagaattgcctccaaatttgggagagctggagagccttacccatctctctctttctttttgtgaaggtatcaagtcccttcctaatagtcttgcaaacctaaccaacttgacaactttggatcttcagtattgcaagtcccttagaaaattgcctccaaatttgaatgttgtacacctcattattaaaggttgctgcagcatcaaggcccttcctacaggtttaagtaacctggccagcttacatctcacacaatgtaactatgatcttgccaatttaaaggactcgctcaacctacgccacctcacccttgagagttgcgaatgtaatgttcacgctgacgttatagaattcctggcaaatttggatgagctgctacaattatctgttgttgatatccaggatacaaaagtcagatatcttccttggagcatcacaaagttactcaatttgaaatttctatgtctccctcagggttttatactcgaaacactaccatatcatctgaatgattccgtcatcatttatatgaaggattgtgacgatcgcaaaacttggaaagaactcaaaacagagattgaaggtaagtgttttcgctattatctcacgaattgttgtttcatgtttgcttctcttccggtaaatagcaaataacaaatagcatagccctctttttatgtcaaaaaacttattcgtaccattgtgcaaacatgggaaggttatatttcaagcattgttgtttcatgctctcctttctatcccaaaaagtttgtttgtcctcctaatccaagtccaaccaattatgcaaataaggaaagattagattcagactatatataataatgttaatatattttcctgttcttcaattttatttcttaattatcttcctctttgtcctcctccagtggataatttgggaatatcaatgtctgtacctcggaacccctcttgttacctttggttggactccaacaagagcctacatccatggctgcagaataattacgattttcaaccgtctgtgaaattcctcgatttaaattttttggatgatgagtttggagatctcacgttgctgaaagagctcacacatgtgacacatctctatatttctggtcatgtagacctctaccgcctccctgacacactcacaaatattacccatctctctcttcatactgaagatgacactgatgattcatttgattcctttcttgataggctggcagagccatcaaacttggtatctttagatctagatcttagtgaaacatacttgccgtcaaacatccatcaattcgtcaaccttaaatgtctcactgtaagatatgccaacagcaagccattagtacctgataactgggaaaagctatctaatttgaaatctttggttctctatacatgttatgatgtatcattgccaacacatttgaatctcactaacctcaagcttttcaattgctttttcgagaatgtcagcttactacctacaagtctacaccgcctagaattattgcatagcaacgactattgcagtgccttttgctgtgatgacggggattgtagtgaagagcctatactatgcttgaatcagtttgtcaacctagagacgctctctataacatgttacgagtacactggcacccgacttcccagcatagcaggactacgcaacttgaaagaattacaacttaaggattgtttcggcctcaaagaattacccccagatttggatgagctagtggaattatccattctcaatatcagcggtaccagagtcaagtcctttcctgattgcatcacaaagctacaaaagttgaaacacgtagtcctgcccaagtgcttcaaaaaggaaaatttacccaataattcaaaaacgaagtacaccactgatgacacggatgaagaatactacaagcatagaggctattatagtagtgaatatgaaacctcaaataaaacctctgatgaaagtaatgagatcacagtagtagattctgcagaggtagccgacaaagtggtttcagaatattcacaggaaggcatcatttcgcagcagatatcatcaccccaactcctgagtatacctaatgctaatcagtttcttggaggtacgtgcttctactatttcagaaatcattgtgtggagtacattgcaattcttctatcttaaaatcaaaatctaattgtcaaatgatcaaggtagtgtgcttccaagttccaacactccttaaccccattaatggggtctaatagagtttgtttcataatattaacttttattgcgtgggtttgaatattaagtttttttatacaaacagatactcatttcactggtagaagcaatacaatgggcgaaagttcacaagttcaagagatggaaacttcatctacaggactcaattcaaatacaaatgaaataaatctcaccgaccagatgttggaattcggatttgggaactcatcatttgattttgggcacatttcttatagtgatgtgactaatattgatcgtgttgagaataaccatcatgcttcagaatatacgcagaacaaagagaatccaccaagtgatgagaaccaggggaagagacagaagaaggagattactcatgagaaaaataatccatgtctgatggatataaacatgacacaagtgcaccttggagaggagctaggcggtacgtttttatcctttacaaagtattttatcagttctcttttgaattcagaagtatatcgggatatgcttactttgactgttgattatcaactatttaaaaagcaaagtttgattttgacaagaataaatgggaactccattaatttagaagattttgcttttggtgcgaatagaatttaatcacaatggaggagaggatgcagtcgatgggatcaatcacaatggaggagaggatgcagtttatgagatcagtcacagcgcttcttgcggttcaccagaccaagacatggagaatatgcctgtaggaaatgataaagagtcaacatccaccatagttggccgagggagaggtaagaaaatagagattaaattgactagagaggaacttcaatcatactggtctagaaacatgacggtagaagatgttgcaaaagacatagatggtatgtttccattctctgcaaactatacggtcattcactgcatttaattgatagatgcatttgatgttctatgattcattccagtgtcaaggtctacatttaaacgctggttgaaggcctccggtattaaatggcaaacaaaacctaattaa

SEQ ID NO: 8 - DNA, 2898 bp, Artificial Sequence
  cDNA of LRR3
atggcagatgaagcaggtaatgtcaactactgttggacgtgttggtcatctattagaaaagtggaagtcgaagtatcccgcatatatgatgacggttacctgttattgaaggaggatccagtggcatggattcaaagtcaccccgctgctgctgatcgtctctctgtgcgaatcttggagttgacattggagctgtatggtgtggataagataacagacatgataggggagctgtctgagctcactcacctctatttctattggtgtctttacctaaagtgtttgcctgacaccatcacaaggctgtccaacttacagttgttaaaacttgtaggttgttatgaattggaagaattaccagaaaatttgggagagctggagagccttacccatctctctctttctcagagtcaagaattgcctccaaatttgggagagctggagagccttacccatctctctctttctttttgtgaaggtatcaagtcccttcctaatagtcttgcaaacctaaccaacttgacaactttggatcttcagtattgcaagtcccttagaaaattgcctccaaatttgaatgttgtacacctcattattaaaggttgctgcagcatcaaggcccttcctacaggtttaagtaacctggccagcttacatctcacacaatgtaactatgatcttgccaatttaaaggactcgctcaacctacgccacctcacccttgagagttgcgaatgtaatgttcacgctgacgttatagaattcctggcaaatttggatgagctgctacaattatctgttgttgatatccaggatacaaaagtcagatatcttccttggagcatcacaaagttactcaatttgaaatttctatgtctccctcagggttttatactcgaaacactaccatatcatctgaatgattccgtcatcatttatatgaaggattgtgacgatcgcaaaacttggaaagaactcaaaacagagattgaagtggataatttgggaatatcaatgtctgtacctcggaacccctcttgttacctttggttggactccaacaagagcctacatccatggctgcagaataattacgattttcaaccgtctgtgaaattcctcgatttaaattttttggatgatgagtttggagatctcacgttgctgaaagagctcacacatgtgacacatctctatatttctggtcatgtagacctctaccgcctccctgacacactcacaaatattacccatctctctcttcatactgaagatgacactgatgattcatttgattcctttcttgataggctggcagagccatcaaacttggtatctttagatctagatcttagtgaaacatacttgccgtcaaacatccatcaattcgtcaaccttaaatgtctcactgtaagatatgccaacagcaagccattagtacctgataactgggaaaagctatctaatttgaaatctttggttctctatacatgttatgatgtatcattgccaacacatttgaatctcactaacctcaagcttttcaattgctttttcgagaatgtcagcttactacctacaagtctacaccgcctagaattattgcatagcaacgactattgcagtgccttttgctgtgatgacggggattgtagtgaagagcctatactatgcttgaatcagtttgtcaacctagagacgctctctataacatgttacgagtacactggcacccgacttcccagcatagcaggactacgcaacttgaaagaattacaacttaaggattgtttcggcctcaaagaattacccccagatttggatgagctagtggaattatccattctcaatatcagcggtaccagagtcaagtcctttcctgattgcatcacaaagctacaaaagttgaaacacgtagtcctgcccaagtgcttcaaaaaggaaaatttacccaataattcaaaaacgaagtacaccactgatgacacggatgaagaatactacaagcatagaggctattatagtagtgaatatgaaacctcaaataaaacctctgatgaaagtaatgagatcacagtagtagattctgcagaggtagccgacaaagtggtttcagaatattcacaggaaggcatcatttcgcagcagatatcatcaccccaactcctgagtatacctaatgctaatcagtttcttggagatactcatttcactggtagaagcaatacaatgggcgaaagttcacaagttcaagagatggaaacttcatctacaggactcaattcaaatacaaatgaaataaatctcaccgaccagatgttggaattcggatttgggaactcatcatttgattttgggcacatttcttatagtgatgtgactaatattgatcgtgttgagaataaccatcatgcttcagaatatacgcagaacaaagagaatccaccaagtgatgagaaccaggggaagagacagaagaaggagattactcatgagaaaaataatccatgtctgatggatataaacatgacacaagtgcaccttggagaggagctaggcgaatttaatcacaatggaggagaggatgcagtcgatgggatcaatcacaatggaggagaggatgcagtttatgagatcagtcacagcgcttcttgcggttcaccagaccaagacatggagaatatgcctgtaggaaatgataaagagtcaacatccaccatagttggccgagggagaggtaagaaaatagagattaaattgactagagaggaacttcaatcatactggtctagaaacatgacggtagaagatgttgcaaaagacatagatgtgtcaaggtctacatttaaacgctggttgaaggcctccggtattaaatggcaaacaaaacctaattaa

SEQ ID NO: 9 - protein, 965 aa, Beta vulgaris
MADEAGNVNYCWTCWSSIRKVEVEVSRIYDDGYLLLKEDPVAWIQSHPAAADRLSVRILELTLELYGVDKITDMIGELSELTHLYFYWCLYLKCLPDTITRLSNLQLLKLVGCYELEELPENLGELESLTHLSLSQSQELPPNLGELESLTHLSLSFCEGIKSLPNSLANLTNLTTLDLQYCKSLRKLPPNLNVVHLIIKGCCSIKALPTGLSNLASLHLTQCNYDLANLKDSLNLRHLTLESCECNVHADVIEFLANLDELLQLSVVDIQDTKVRYLPWSITKLLNLKFLCLPQGFILETLPYHLNDSVIIYMKDCDDRKTWKELKTEIEVDNLGISMSVPRNPSCYLWLDSNKSLHPWLQNNYDFQPSVKFLDLNFLDDEFGDLTLLKELTHVTHLYISGHVDLYRLPDTLTNITHLSLHTEDDTDDSFDSFLDRLAEPSNLVSLDLDLSETYLPSNIHQFVNLKCLTVRYANSKPLVPDNWEKLSNLKSLVLYTCYDVSLPTHLNLTNLKLFNCFFENVSLLPTSLHRLELLHSNDYCSAFCCDDGDCSEEPILCLNQFVNLETLSITCYEYTGTRLPSIAGLRNLKELQLKDCFGLKELPPDLDELVELSILNISGTRVKSFPDCITKLQKLKHVVLPKCFKKENLPNNSKTKYTTDDTDEEYYKHRGYYSSEYETSNKTSDESNEITVVDSAEVADKVVSEYSQEGIISQQISSPQLLSIPNANQFLGDTHFTGRSNTMGESSQVQEMETSSTGLNSNTNEINLTDQMLEFGFGNSSFDFGHISYSDVTNIDRVENNHHASEYTQNKENPPSDENQGKRQKKEITHEKNNPCLMDINMTQVHLGEELGEFNHNGGEDAVDGINHNGGEDAVYEISHSASCGSPDQDMENMPVGNDKESTSTIVGRGRGKKIEIKLTREELQSYWSRNMTVEDVAKDIDVSRSTFKRWLKASGIKWQTKPN

SEQ ID NO: 10 - DNA, 201 bp, Artificial Sequence
  marker s5e3001s02; resistant allele prefrably T
mtttccttaaaccctaaaccctarttaatatgttcacatttttctrctaattagatctgaataacttatgccttttattttatttttgttgttgtttattkatgatttcaggattttratttggtgatgatatcagaaagtaattctctttttgattgattgagaatttaaktttatagaatttgaagatggcgtataggc

SEQ ID NO: 11 - DNA, 201 bp, Artificial Sequence
  marker s5e4668xxx; resistant allele preferably T
gtggcctgcctttagtcggctatctcccttttctgggttctaatctccatcatagcttcaaagaattggccagtttatatggtccaatcttcaaactccgkcttggaactaaagattgtattgtgatcacctcaccatcacttgtcaaggaggtggttagggaccaagatgttgtgttcgctaaccgaggacacattattg